European Patent Specification EP 3 626 264 B1, published August 23, 2023. Title: RECOMBINANT RESPIRATORY SYNCYTIAL VIRUS G PROTEIN FRAGMENTS. Applicant: THE UNITED STATES OF AMERICA, AS REPRESENTED BY THE SECRETARY, DEPARTMENT OF HEALTH AND HUMAN SERVICES. The sequence listing filed with the application follows.

SEQUENCE LISTING (9 sequences)

SEQ ID NO: 1 - DNA, 696 bp, Artificial Sequence
  source: /note="Description of Artificial Sequence: Synthetic polynucleotide"
cataaagtcaccccgaccacggcgattatccaggatgccacctctcaaatcaaaaacaccacgccgacgtacctgacccagaatccgcaactgggcatttcaccgtcgaacccgtcagaaatcacctcgcagattaccacgatcctggcaagcaccacgccgggtgtcaaaagcacgctgcaatctaccacggtgaaaaccaaaaataccacgaccacgcagacccaaccgagcaaaccgaccacgaaacagcgtcaaaataaaccgccgtctaaaccgaacaatgattttcacttcgaagtgtttaacttcgttccgtgcagtatttgttccaacaatccgacctgctgggccatttgtaaacgcatcccgaacaaaaaaccgggcaagaaaaccacgaccaaaccgacgaaaaaaccgaccctgaaaacgaccaaaaaagacccgaaaccgcagacgaccaaaagcaaagaagtgccgacgaccaaaccgacggaagaaccgaccattaacacgaccaaaaccaatattatcacgaccctgctgacctccaacacgaccggcaatccggaactgacctcacagatggaaacgttccattcgaccagctctgaaggtaatccgagcccgtctcaggtcagcacgacctccgaatacccgagccagccgtcttctccgccgaataccccgcgtcag

SEQ ID NO: 2 - protein, 232 aa, Artificial Sequence
  source: /note="Description of Artificial Sequence: Synthetic polypeptide"
HKVTPTTAIIQDATSQIKNTTPTYLTQNPQLGISPSNPSEITSQITTILASTTPGVKSTLQSTTVKTKNTTTTQTQPSKPTTKQRQNKPPSKPNNDFHFEVFNFVPCSICSNNPTCWAICKRIPNKKPGKKTTTKPTKKPTLKTTKKDPKPQTTKSKEVPTTKPTEEPTINTTKTNIITTLLTSNTTGNPELTSQMETFHSTSSEGNPSPSQVSTTSEYPSQPSSPPNTPRQ

SEQ ID NO: 3 - DNA, 696 bp, Artificial Sequence
  source: /note="Description of Artificial Sequence: Synthetic polynucleotide"
cacaaagtcacaccaacaactgcaatcatacaagatgcaacaagccagatcaagaacacaaccccaacatacctcacccagaatcctcagcttggaatcagtccctctaatccgtctgaaattacatcacaaatcaccaccatactagcttcaacaacaccaggagtcaagtcaaccctgcaatccacaacagtcaagaccaaaaacacaacaacaactcaaacacaacccagcaagcccaccacaaaacaacgccaaaacaaaccaccaagcaaacccaataatgattttcactttgaagtgttcaactttgtaccctgcagcatatgcagcaacaatccaacctgctgggctatctgcaaaagaataccaaacaaaaaaccaggaaagaaaaccactaccaagcccacaaaaaaaccaaccctcaagacaaccaaaaaagatcccaaacctcaaaccactaaatcaaaggaagtacccaccaccaagcccacagaagagccaaccatcaacaccaccaaaacaaacatcataactacactactcacctccaacaccacaggaaatccagaactcacaagtcaaatggaaaccttccactcaacttcctccgaaggcaatccaagcccttctcaagtctctacaacatccgagtacccatcacaaccttcatctccacccaacacaccacgccag

SEQ ID NO: 4 - protein, 298 aa, Respiratory syncytial virus
MSKNKDQRTAKTLERTWDTLNHLLFISSCLYKLNLKSVAQITLSILAMIISTSLIIAAIIFIASANHKVTPTTAIIQDATSQIKNTTPTYLTQNPQLGISPSNPSEITSQITTILASTTPGVKSTLQSTTVKTKNTTTTQTQPSKPTTKQRQNKPPSKPNNDFHFEVFNFVPCSICSNNPTCWAICKRIPNKKPGKKTTTKPTKKPTLKTTKKDPKPQTTKSKEVPTTKPTEEPTINTTKTNIITTLLTSNTTGNPELTSQMETFHSTSSEGNPSPSQVSTTSEYPSQPSSPPNTPRQ

SEQ ID NO: 5 - protein, 298 aa, Respiratory syncytial virus
MSKNKDQRTAKTLEKTWDTLNHLLFISSGLYKLNLKSIAQITLSILAMIISTSLIITAIIFIASANHKVTLTTAIIQDATSQIKNTTPTYLTQDPQLGISFSNLSEITSQTTTILASTTPGVKSNLQPTTVKTKNTTTTQTQPSKPTTKQRQNKPPNKPNNDFHFEVFNFVPCSICSNNPTCWAICKRIPNKKPGKKTTTKPTKKPTFKTTKKDHKPQTTKPKEVPTTKPTEEPTINTTKTNIITTLLTNNTTGNPKLTSQMETFHSTSSEGNLSPSQVSTTSEHPSQPSSPPNTTRQ

SEQ ID NO: 6 - protein, 292 aa, Respiratory syncytial virus
MSKHKNQRTARTLEKTWDTLNHLIVISSCLYRLNLKSIAQIALSVLAMIISTSLIIAAIIFIISANHKVTLTTVTVQTIKNHTEKNISTYLTQVPPERVNSSKQPTTTSPIHTNSATISPNTKSETHHTTAQTKGRITTSTQTNKPSTKSRSKNPPKKPKDDYHFEVFNFVPCSICGNNQLCKSICKTIPSNKPKKKPTIKPTNKPTTKTTNKRDPKTPAKMPKKEIITNPAKKPTLKTTERDTSISQSTVLDTITPKYTIQQQSLHSTTSENTPSSTQIPTASEPSTLNPN

SEQ ID NO: 7 - protein, 299 aa, Respiratory syncytial virus
MSKHKNQRTARTLEKTWDTLNHLIVISSCLYRLNLKSIAQIALSVLAMIISTSLIIAAIIFIISANHKVTLTTVTVQTIKNHTEKNITTYLTQVPPERVSSSKQPTTTSPIHTNSATTSPNTKSETHHTTAQTKGRTTTSTQTNKPSTKPRLKNPPKKPKDDYHFEVFNFVPCSICGNNQLCKSICKTIPSNKPKKKPTIKPTNKPTTKTTNKRDPKTPAKTTKKETTTNPTKKPTLTTTERDTSTSQSTVLDTTTLEHTIQQQSLHSTTPENTPNSTQTPTASEPSTSNSTQNTQSHA

SEQ ID NO: 8 - protein, 6 aa, Artificial Sequence
  source: /note="Description of Artificial Sequence: Synthetic 6xHis tag"
HHHHHH

SEQ ID NO: 9 - protein, 23 aa, Respiratory syncytial virus
HFEVFNFVPCSICSNNPTCWAIC